European Patent Application EP 4 707 403 A2, published March 11, 2026. Title: METHOD RELATING TO MYOSTATIN PATHWAY INHIBITION. Applicant: UCL BUSINESS PLC. Application WO PCT/GB2018/050619, filed March 12, 2018. The sequence listing filed with the application follows.

SEQUENCE LISTING (42 sequences)

SEQ ID NO: 1 - DNA, 20 bp, synthetic construct
  misc_feature 1..20: note = Primer
  source 1..20: mol_type = other DNA
ctggctcctagcaccatgaa

SEQ ID NO: 2 - DNA, 20 bp, synthetic construct
  misc_feature 1..20: note = Primer
  source 1..20: mol_type = other DNA
ctgcttgctgatccacatct

SEQ ID NO: 3 - DNA, 20 bp, synthetic construct
  misc_feature 1..20: note = Primer
  source 1..20: mol_type = other DNA
ccttcattggaaacagcaca

SEQ ID NO: 4 - DNA, 20 bp, synthetic construct
  misc_feature 1..20: note = Primer
  source 1..20: mol_type = other DNA
cctcctctccgaaatcctct

SEQ ID NO: 5 - DNA, 20 bp, synthetic construct
  misc_feature 1..20: note = Primer
  source 1..20: mol_type = other DNA
ttgtgatgggtgtgaaccac

SEQ ID NO: 6 - DNA, 20 bp, synthetic construct
  misc_feature 1..20: note = Primer
  source 1..20: mol_type = other DNA
ttcagctctgggatgacctt

SEQ ID NO: 7 - DNA, 20 bp, synthetic construct
  misc_feature 1..20: note = Primer
  source 1..20: mol_type = other DNA
gcaaactttgctttccctgg

SEQ ID NO: 8 - DNA, 22 bp, synthetic construct
  misc_feature 1..22: note = Primer
  source 1..22: mol_type = other DNA
acttcgagaggtccttttcacc

SEQ ID NO: 9 - DNA, 20 bp, synthetic construct
  misc_feature 1..20: note = Primer
  source 1..20: mol_type = other DNA
ctccaagcagatgcagcaga

SEQ ID NO: 10 - DNA, 19 bp, synthetic construct
  misc_feature 1..19: note = Primer
  source 1..19: mol_type = other DNA
atagccttgcgcatcatgg

SEQ ID NO: 11 - DNA, 19 bp, synthetic construct
  misc_feature 1..19: note = Primer
  source 1..19: mol_type = other DNA
gctcagctcatgaacgact

SEQ ID NO: 12 - DNA, 19 bp, synthetic construct
  misc_feature 1..19: note = Primer
  source 1..19: mol_type = other DNA
ctctgccacgactgcttgt

SEQ ID NO: 13 - DNA, 21 bp, synthetic construct
  misc_feature 1..21: note = Primer
  source 1..21: mol_type = other DNA
ctcttcaagtggatgattttc

SEQ ID NO: 14 - DNA, 21 bp, synthetic construct
  misc_feature 1..21: note = Primer
  source 1..21: mol_type = other DNA
acagtaggcattattggtctg

SEQ ID NO: 15 - DNA, 21 bp, synthetic construct
  misc_feature 1..21: note = Primer
  source 1..21: mol_type = other DNA
gcactggtatttggcagagta

SEQ ID NO: 16 - DNA, 21 bp, synthetic construct
  misc_feature 1..21: note = Primer
  source 1..21: mol_type = other DNA
cacactctcctgagcagtaat

SEQ ID NO: 17 - DNA, 20 bp, synthetic construct
  misc_feature 1..20: note = Primer
  source 1..20: mol_type = other DNA
ctctctttctggcctggagg

SEQ ID NO: 18 - DNA, 22 bp, synthetic construct
  misc_feature 1..22: note = Primer
  source 1..22: mol_type = other DNA
tgctggatgacgtgagtaaacc

SEQ ID NO: 19 - DNA, 23 bp, synthetic construct
  misc_feature 1..23: note = Primer
  source 1..23: mol_type = other DNA
aaggtgaaggtcggagtcaacgg

SEQ ID NO: 20 - DNA, 23 bp, synthetic construct
  misc_feature 1..23: note = Primer
  source 1..23: mol_type = other DNA
tgacaagcttcccgttctcagcc

SEQ ID NO: 21 - DNA, 22 bp, synthetic construct
  misc_feature 1..22: note = Primer
  source 1..22: mol_type = other DNA
ctcatttggaattttgccgatt

SEQ ID NO: 22 - DNA, 22 bp, synthetic construct
  misc_feature 1..22: note = Primer
  source 1..22: mol_type = other DNA
ccgagtgaagatccccttttta

SEQ ID NO: 23 - DNA, 22 bp, synthetic construct
  misc_feature 1..22: note = Primer
  source 1..22: mol_type = other DNA
tccaggctttaggtatcaccac

SEQ ID NO: 24 - DNA, 21 bp, synthetic construct
  misc_feature 1..21: note = Primer
  source 1..21: mol_type = other DNA
gctcccactttgtctccagtc

SEQ ID NO: 25 - DNA, 20 bp, synthetic construct
  misc_feature 1..20: note = Primer
  source 1..20: mol_type = other DNA
cctaaagcatacgggtcctg

SEQ ID NO: 26 - DNA, 20 bp, synthetic construct
  misc_feature 1..20: note = Primer
  source 1..20: mol_type = other DNA
tttcactttgccaaacacca

SEQ ID NO: 27 - DNA, 19 bp, synthetic construct
  misc_feature 1..19: note = Primer
  source 1..19: mol_type = other DNA
ctcctctggggatcgctgt

SEQ ID NO: 28 - DNA, 20 bp, synthetic construct
  misc_feature 1..20: note = Primer
  source 1..20: mol_type = other DNA
ctcccagttggcgttgtagt

SEQ ID NO: 29 - DNA, 17 bp, synthetic construct
  misc_feature 1..17: note = Primer
  source 1..17: mol_type = other DNA
cggctgagcacctcgtg

SEQ ID NO: 30 - DNA, 20 bp, synthetic construct
  misc_feature 1..20: note = Primer
  source 1..20: mol_type = other DNA
ttcttgttcattcggcattt

SEQ ID NO: 31 - DNA, 20 bp, synthetic construct
  misc_feature 1..20: note = Primer
  source 1..20: mol_type = other DNA
ttttacccaaagctcctcca

SEQ ID NO: 32 - DNA, 20 bp, synthetic construct
  misc_feature 1..20: note = Primer
  source 1..20: mol_type = other DNA
gagtctcgacgggtctcaaa

SEQ ID NO: 33 - DNA, 20 bp, synthetic construct
  misc_feature 1..20: note = Primer
  source 1..20: mol_type = other DNA
cacacttctgcacgctccac

SEQ ID NO: 34 - DNA, 19 bp, synthetic construct
  misc_feature 1..19: note = Primer
  source 1..19: mol_type = other DNA
tttgccgagtcaggcacag

SEQ ID NO: 35 - DNA, 20 bp, synthetic construct
  misc_feature 1..20: note = Primer
  source 1..20: mol_type = other DNA
atcagccgggaggtagtgaa

SEQ ID NO: 36 - DNA, 21 bp, synthetic construct
  misc_feature 1..21: note = Primer
  source 1..21: mol_type = other DNA
ctgggccatgcttatgaccgt

SEQ ID NO: 37 - DNA, 20 bp, synthetic construct
  misc_feature 1..20: note = Primer
  source 1..20: mol_type = other DNA
ttatggagcagacctcggag

SEQ ID NO: 38 - DNA, 20 bp, synthetic construct
  misc_feature 1..20: note = Primer
  source 1..20: mol_type = other DNA
aaatctcgaagtgcagcgtc

SEQ ID NO: 39 - DNA, 20 bp, synthetic construct
  misc_feature 1..20: note = Primer
  source 1..20: mol_type = other DNA
attggcagagcatcgacttc

SEQ ID NO: 40 - DNA, 21 bp, synthetic construct
  misc_feature 1..21: note = Primer
  source 1..21: mol_type = other DNA
ttttgtgttctctaggactcg

SEQ ID NO: 41 - DNA, 21 bp, synthetic construct
  misc_feature 1..21: note = Primer
  source 1..21: mol_type = other DNA
gcaatgaagagctgaatgcca

SEQ ID NO: 42 - DNA, 21 bp, synthetic construct
  misc_feature 1..21: note = Primer
  source 1..21: mol_type = other DNA
tgtcaaagacacgcagaccct